European Patent Application EP 4 144 857 A1, published March 8, 2023. Title: ANIMAL PREPARATION METHOD. Applicant: MINGCELER BIOTECHNOLOGY CO., LTD. Application EP20923578.7. The sequence listing filed with the application follows.

SEQUENCE LISTING (32 sequences)

SEQ ID NO: 1 - DNA, 23 bp, Natural sequence
  sgRNA1 sequence
tactgctcagtccctcaccgagg

SEQ ID NO: 2 - DNA, 23 bp, Natural sequence
  sgRNA2sequence
cttggcattttcctcggtgaggg

SEQ ID NO: 3 - DNA, 23 bp, Natural sequence
  sgRNRA3sequence
caagtgaactttgataagacagg

SEQ ID NO: 4 - DNA, 25 bp, Artificial Sequence
  Upstream primer for synthesizing sgRNA1
caccgcttggcattttcctcggtga

SEQ ID NO: 5 - DNA, 25 bp, Artificial Sequence
  Downstream primer for synthesizing sgRNA1
aaactcaccgaggaaaatgccaagc

SEQ ID NO: 6 - DNA, 25 bp, Artificial Sequence
  Upstream primer for synthesizing sgRNA2
caccgtactgctcagtccctcaccg

SEQ ID NO: 7 - DNA, 25 bp, Artificial Sequence
  Downstream primer for synthesizing sgRNA2
aaaccggtgagggactgagcagtac

SEQ ID NO: 8 - DNA, 25 bp, Artificial Sequence
  Upstream primer for synthesizing sgRNA3
caccgcaagtgaactttgataagac

SEQ ID NO: 9 - DNA, 25 bp, Artificial Sequence
  Downstream primer for synthesizing sgRNA3
aaacgtcttatcaaagttcacttgc

SEQ ID NO: 10 - DNA, 28 bp, Natural sequence
  5arm-sgF
ggttttgatttggccataaaatgttagc

SEQ ID NO: 11 - DNA, 25 bp, Natural sequence
  3arm-sgR
attcccaggtccagtttcacctaag

SEQ ID NO: 12 - DNA, 2418 bp, Natural sequence
  hACE2-CDS
atgtcaagctcttcctggctccttctcagccttgttgctgtaactgctgctcagtccaccattgaggaacaggccaagacatttttggacaagtttaaccacgaagccgaagacctgttctatcaaagttcacttgcttcttggaattataacaccaatattactgaagagaatgtccaaaacatgaataatgctggggacaaatggtctgcctttttaaaggaacagtccacacttgcccaaatgtatccactacaagaaattcagaatctcacagtcaagcttcagctgcaggctcttcagcaaaatgggtcttcagtgctctcagaagacaagagcaaacggttgaacacaattctaaatacaatgagcaccatctacagtactggaaaagtttgtaacccagataatccacaagaatgcttattacttgaaccaggtttgaatgaaataatggcaaacagtttagactacaatgagaggctctgggcttgggaaagctggagatctgaggtcggcaagcagctgaggccattatatgaagagtatgtggtcttgaaaaatgagatggcaagagcaaatcattatgaggactatggggattattggagaggagactatgaagtaaatggggtagatggctatgactacagccgcggccagttgattgaagatgtggaacatacctttgaagagattaaaccattatatgaacatcttcatgcctatgtgagggcaaagttgatgaatgcctatccttcctatatcagtccaattggatgcctccctgctcatttgcttggtgatatgtggggtagattttggacaaatctgtactctttgacagttccctttggacagaaaccaaacatagatgttactgatgcaatggtggaccaggcctgggatgcacagagaatattcaaggaggccgagaagttctttgtatctgttggtcttcctaatatgactcaaggattctgggaaaattccatgctaacggacccaggaaatgttcagaaagcagtctgccatcccacagcttgggacctggggaagggcgacttcaggatccttatgtgcacaaaggtgacaatggacgacttcctgacagctcatcatgagatggggcatatccagtatgatatggcatatgctgcacaaccttttctgctaagaaatggagctaatgaaggattccatgaagctgttggggaaatcatgtcactttctgcagccacacctaagcatttaaaatccattggtcttctgtcacccgattttcaagaagacaatgaaacagaaataaacttcctgctcaaacaagcactcacgattgttgggactctgccatttacttacatgttagagaagtggaggtggatggtctttaaaggggaaattcccaaagaccagtggatgaaaaagtggtgggagatgaagcgagagatagttggggtggtggaacctgtgccccatgatgaaacatactgtgaccccgcatctctgttccatgtttctaatgattactcattcattcgatattacacaaggaccctttaccaattccagtttcaagaagcactttgtcaagcagctaaacatgaaggccctctgcacaaatgtgacatctcaaactctacagaagctggacagaaactgttcaatatgctgaggcttggaaaatcagaaccctggaccctagcattggaaaatgttgtaggagcaaagaacatgaatgtaaggccactgctcaactactttgagcccttatttacctggctgaaagaccagaacaagaattcttttgtgggatggagtaccgactggagtccatatgcagaccaaagcatcaaagtgaggataagcctaaaatcagctcttggagataaagcatatgaatggaacgacaatgaaatgtacctgttccgatcatctgttgcatatgctatgaggcagtactttttaaaagtaaaaaatcagatgattctttttggggaggaggatgtgcgagtggctaatttgaaaccaagaatctcctttaatttctttgtcactgcacctaaaaatgtgtctgatatcattcctagaactgaagttgaaaaggccatcaggatgtcccggagccgtatcaatgatgctttccgtctgaatgacaacagcctagagtttctggggatacagccaacacttggacctcctaaccagccccctgtttccatatggctgattgtttttggagttgtgatgggagtgatagtggttggcattgtcatcctgatcttcactgggatcagagatcggaagaagaaaaataaagcaagaagtggagaaaatccttatgcctccatcgatattagcaaaggagaaaataatccaggattccaaaacactgatgatgttcagacctccttttag

SEQ ID NO: 13 - protein, 805 aa, Natural sequence [sequence omitted]

SEQ ID NO: 14 - DNA, 122 bp, Natural sequence
  SV40 polyA
aacttgtttattgcagcttataatggttacaaataaagcaatagcatcacaaatttcacaaataaagcatttttttcactgcattctagttgtggtttgtccaaactcatcaatgtatctta

SEQ ID NO: 15 - DNA, 970 bp, Natural sequence
  5¡¯ homology arm
ccctatggagtggagaagagtcttataattttttaaatgggcagagaaatgaatttatttttaatttttagagacagggtttctttgtatagctctagctgtctttgattggtagacaaagctgtcctcaaactcagagatcttccttcctttgtctcctgagtgctgggattaaaggcatggaccaccactgccctgccccattctctccattaattttaagtgaatgcttgcaaaagctcacttctttggtgaacagcttcctttacaaataagtacctttgccttcgtttttataggattcttaaaaagaaaaaaaagattcagccaggtggttgtggtgcacacctttaatcccagcagtcaggaggcagaggaaagcagatctcttgagtttgaggctagcctagtctacagagggagttccaggacagccaaggctacagagaggaactgtctaaaaacaccaagaaagagagaaaggagagagggagaggatggatagcttattgatagaattgtcagaaaaggctataagttccaatatgtgtcccatgatttctaagtctagccctttctgttatagtaaaatcatagtacaccctcctcctccagtgtatctttaacagcttttaaggaacatattaactaaatgtccaggttttgatttggccataaaatgttagcaaagctaaggttttctaggattaatgaataacatgtctttatttagtttacttaaaaaaatcattctaaaatatctgtttacatatctgtcctctccaggattaacttcatattggtccagcagcttgtttactgttctcttctgtttcttcttctgctttttttttcttctcttctcagtgcccaacccaagttcaaaggctgatgagagagaaaaactcatgaagagattttactctagggaaagttgctcagtggatgggatcttggcgcacggggaaag

SEQ ID NO: 16 - DNA, 971 bp, Natural sequence
  3¡¯ homology arm
gaattataatactaacattactgaagaaaatgcccaaaagatggtaagttcttgaggctacccagggggttattgattgcttcttaaagatcagaattactgcctataaaactggataaggaaatcatagagatctctcaagtgtgaggatgagtgactgcctctgtagctctgatcctagtctcccagatggctaaattcaattgaccttagagttcatctggaaaattgttatgaatgaattatttgcccagattccaaagatgagtgaaaatgtttaataaagttgccatcactattctcattatatttggtatgtaaagcattcatggaaatgttctaagtcgttattgagccaataattttctttagcttataatgccaacaggtctatccgagaactacaaatgacatattaactgaaaaatgcaactggggtttactgaaggcagcagcttagtaattaaggtaaccatggcttaggtgaaactggacctgggaattccttctttcattgacacagagctctgaggaatttccaaaggtcacagaagaaaagctataattaaactagtcccaaaaaatctcagcctactctgggaaagcagcatattttgtttgacaagtgcaaggacttagaacttttttttttctcactgatcctgaagtgccttttaagtatagttaagtggtggaaaattgagcaactatttaagaaaagactcttttttttcttcttccagcaatgctttccttcaaaacggtagcttcaaaacttcctgtcttttaaatgatcagggggctgtgtgtttaaattattgccattcatagaacagagtgggtctgaggatgcctgtttcctttgaaattctatgccccctcccagttttctaaaatttaagaaaccacagagactttgacaatgtagttgccaaatgagttgcttttaactgctctaatagtttggtctt

SEQ ID NO: 17 - DNA, 1124 bp, Artificial Sequence
  PGK-puro
gggtaggggaggcgcttttcccaaggcagtctggagcatgcgctttagcagccccgctgggcacttggcgctacacaagtggcctctggcctcgcacacattccacatcccccggtaggcgccaaccggctccgttctttggtggccccttcgcgccaccttctactcctcccctagtcaggaagttcccccccgccccgcagctcgcgtcgtgcaggacgtgacaaatggaagtagcacgtctcactagtctcgtgcagatggacagcaccgctgagcaatggaagcgggtaggcctttggggcagcggccaatagcagctttgctccttcgctttctgggctcagaggctgggaaggggtgggtccgggggcgggctcaggggcgggctcaggggcggggcgggcgcccgaaggtcctccggaggcccggcattctgcacgcttcaaaagcgcacgtctgccgcgctgttctcctcttcctcatctccgggcctttcgacctgcagcccaagctagcttaccatgaccgagtacaagcccacggtgcgcctcgccacccgcgacgacgtccccagggccgtacgcaccctcgccgccgcgttcgccgactaccccgccacgcgccacaccgtcgatccggaccgccacatcgagcgggtcaccgagctgcaagaactcttcctcacgcgcgtcgggctcgacatcggcaaggtgtgggtcgcggacgacggcgccgcggtggcggtctggaccacgccggagagcgtcgaagcgggggcggtgttcgccgagatcggcccgcgcatggccgagttgagcggttcccggctggccgcgcagcaacagatggaaggcctcctggcgccgcaccggcccaaggagcccgcgtggttcctggccaccgtcggcgtctcgcccgaccaccagggcaagggtctgggcagcgccgtcgtgctccccggagtggaggcggccgagcgcgccggggtgcccgccttcctggagacctccgcgccccgcaacctccccttctacgagcggctcggcttcaccgtcaccgccgacgtcgaggtgcccgaaggaccgcgcacctggtgcatgacccgcaagcccggtgcctga

SEQ ID NO: 18 - DNA, 34 bp, Natural sequence
  Frt
gaagttcctattctctagaaagtataggaacttc

SEQ ID NO: 19 - DNA, 50 bp, Artificial Sequence
  5arm-pcrF
tcgcacacattccacatccaccggtccctatggagtggagaagagtctta

SEQ ID NO: 20 - DNA, 47 bp, Artificial Sequence
  5arm-pcrR
gaaggagccaggaagagcttgacatctttccccgtgcgccaagatcc

SEQ ID NO: 21 - DNA, 47 bp, Artificial Sequence
  hACE2-F
ggatcttggcgcacggggaaagatgtcaagctcttcctggctccttc

SEQ ID NO: 22 - DNA, 49 bp, Artificial Sequence
  hACE2-R
cattataagctgcaataaacaagttctaaaaggaggtctgaacatcatc

SEQ ID NO: 23 - DNA, 49 bp, Artificial Sequence
  SV40-F
gatgatgttcagacctccttttagaacttgtttattgcagcttataatg

SEQ ID NO: 24 - DNA, 48 bp, Artificial Sequence
  SV40-R
agagaataggaacttcgcacgcgttaagatacattgatgagtttggac

SEQ ID NO: 25 - DNA, 50 bp, Artificial Sequence
  3arm-pcrF
tacgaagttatgtcgacgcggcgcgccgaattataatactaacattactg

SEQ ID NO: 26 - DNA, 53 bp, Artificial Sequence
  3arm-pcrR
tatgaccatgattacgccaagcttaagaccaaactattagagcagttaaaagc

SEQ ID NO: 27 - DNA, 8470 bp, Artificial Sequence
  Targeting vector
tcgcgcgtttcggtgatgacggtgaaaacctctgacacatgcagctcccggagacggtcacagcttgtctgtaagcggatgccgggagcagacaagcccgtcagggcgcgtcagcgggtgttggcgggtgtcggggctggcttaactatgcggcatcagagcagattgtactgagagtgcaccatatgtaccgggtaggggaggcgcttttcccaaggcagtctggagcatgcgctttagcagccccgctgggcacttggcgctacacaagtggcctctggcctcgcacacattccacatccaccggtccctatggagtggagaagagtcttataattttttaaatgggcagagaaatgaatttatttttaatttttagagacagggtttctttgtatagctctagctgtctttgattggtagacaaagctgtcctcaaactcagagatcttccttcctttgtctcctgagtgctgggattaaaggcatggaccaccactgccctgccccattctctccattaattttaagtgaatgcttgcaaaagctcacttctttggtgaacagcttcctttacaaataagtacctttgccttcgtttttataggattcttaaaaagaaaaaaaagattcagccaggtggttgtggtgcacacctttaatcccagcagtcaggaggcagaggaaagcagatctcttgagtttgaggctagcctagtctacagagggagttccaggacagccaaggctacagagaggaactgtctaaaaacaccaagaaagagagaaaggagagagggagaggatggatagcttattgatagaattgtcagaaaaggctataagttccaatatgtgtcccatgatttctaagtctagccctttctgttatagtaaaatcatagtacaccctcctcctccagtgtatctttaacagcttttaaggaacatattaactaaatgtccaggttttgatttggccataaaatgttagcaaagctaaggttttctaggattaatgaataacatgtctttatttagtttacttaaaaaaatcattctaaaatatctgtttacatatctgtcctctccaggattaacttcatattggtccagcagcttgtttactgttctcttctgtttcttcttctgctttttttttcttctcttctcagtgcccaacccaagttcaaaggctgatgagagagaaaaactcatgaagagattttactctagggaaagttgctcagtggatgggatcttggcgcacggggaaagatgtcaagctcttcctggctccttctcagccttgttgctgtaactgctgctcagtccaccattgaggaacaggccaagacatttttggacaagtttaaccacgaagccgaagacctgttctatcaaagttcacttgcttcttggaattataacaccaatattactgaagagaatgtccaaaacatgaataatgctggggacaaatggtctgcctttttaaaggaacagtccacacttgcccaaatgtatccactacaagaaattcagaatctcacagtcaagcttcagctgcaggctcttcagcaaaatgggtcttcagtgctctcagaagacaagagcaaacggttgaacacaattctaaatacaatgagcaccatctacagtactggaaaagtttgtaacccagataatccacaagaatgcttattacttgaaccaggtttgaatgaaataatggcaaacagtttagactacaatgagaggctctgggcttgggaaagctggagatctgaggtcggcaagcagctgaggccattatatgaagagtatgtggtcttgaaaaatgagatggcaagagcaaatcattatgaggactatggggattattggagaggagactatgaagtaaatggggtagatggctatgactacagccgcggccagttgattgaagatgtggaacatacctttgaagagattaaaccattatatgaacatcttcatgcctatgtgagggcaaagttgatgaatgcctatccttcctatatcagtccaattggatgcctccctgctcatttgcttggtgatatgtggggtagattttggacaaatctgtactctttgacagttccctttggacagaaaccaaacatagatgttactgatgcaatggtggaccaggcctgggatgcacagagaatattcaaggaggccgagaagttctttgtatctgttggtcttcctaatatgactcaaggattctgggaaaattccatgctaacggacccaggaaatgttcagaaagcagtctgccatcccacagcttgggacctggggaagggcgacttcaggatccttatgtgcacaaaggtgacaatggacgacttcctgacagctcatcatgagatggggcatatccagtatgatatggcatatgctgcacaaccttttctgctaagaaatggagctaatgaaggattccatgaagctgttggggaaatcatgtcactttctgcagccacacctaagcatttaaaatccattggtcttctgtcacccgattttcaagaagacaatgaaacagaaataaacttcctgctcaaacaagcactcacgattgttgggactctgccatttacttacatgttagagaagtggaggtggatggtctttaaaggggaaattcccaaagaccagtggatgaaaaagtggtgggagatgaagcgagagatagttggggtggtggaacctgtgccccatgatgaaacatactgtgaccccgcatctctgttccatgtttctaatgattactcattcattcgatattacacaaggaccctttaccaattccagtttcaagaagcactttgtcaagcagctaaacatgaaggccctctgcacaaatgtgacatctcaaactctacagaagctggacagaaactgttcaatatgctgaggcttggaaaatcagaaccctggaccctagcattggaaaatgttgtaggagcaaagaacatgaatgtaaggccactgctcaactactttgagcccttatttacctggctgaaagaccagaacaagaattcttttgtgggatggagtaccgactggagtccatatgcagaccaaagcatcaaagtgaggataagcctaaaatcagctcttggagataaagcatatgaatggaacgacaatgaaatgtacctgttccgatcatctgttgcatatgctatgaggcagtactttttaaaagtaaaaaatcagatgattctttttggggaggaggatgtgcgagtggctaatttgaaaccaagaatctcctttaatttctttgtcactgcacctaaaaatgtgtctgatatcattcctagaactgaagttgaaaaggccatcaggatgtcccggagccgtatcaatgatgctttccgtctgaatgacaacagcctagagtttctggggatacagccaacacttggacctcctaaccagccccctgtttccatatggctgattgtttttggagttgtgatgggagtgatagtggttggcattgtcatcctgatcttcactgggatcagagatcggaagaagaaaaataaagcaagaagtggagaaaatccttatgcctccatcgatattagcaaaggagaaaataatccaggattccaaaacactgatgatgttcagacctccttttagaacttgtttattgcagcttataatggttacaaataaagcaatagcatcacaaatttcacaaataaagcatttttttcactgcattctagttgtggtttgtccaaactcatcaatgtatcttaacgcgtgcgaagttcctattctctagaaagtataggaacttcatcgataccgggtaggggaggcgcttttcccaaggcagtctggagcatgcgctttagcagccccgctgggcacttggcgctacacaagtggcctctggcctcgcacacattccacatcccccggtaggcgccaaccggctccgttctttggtggccccttcgcgccaccttctactcctcccctagtcaggaagttcccccccgccccgcagctcgcgtcgtgcaggacgtgacaaatggaagtagcacgtctcactagtctcgtgcagatggacagcaccgctgagcaatggaagcgggtaggcctttggggcagcggccaatagcagctttgctccttcgctttctgggctcagaggctgggaaggggtgggtccgggggcgggctcaggggcgggctcaggggcggggcgggcgcccgaaggtcctccggaggcccggcattctgcacgcttcaaaagcgcacgtctgccgcgctgttctcctcttcctcatctccgggcctttcgacctgcagcccaagctagcttaccatgaccgagtacaagcccacggtgcgcctcgccacccgcgacgacgtccccagggccgtacgcaccctcgccgccgcgttcgccgactaccccgccacgcgccacaccgtcgatccggaccgccacatcgagcgggtcaccgagctgcaagaactcttcctcacgcgcgtcgggctcgacatcggcaaggtgtgggtcgcggacgacggcgccgcggtggcggtctggaccacgccggagagcgtcgaagcgggggcggtgttcgccgagatcggcccgcgcatggccgagttgagcggttcccggctggccgcgcagcaacagatggaaggcctcctggcgccgcaccggcccaaggagcccgcgtggttcctggccaccgtcggcgtctcgcccgaccaccagggcaagggtctgggcagcgccgtcgtgctccccggagtggaggcggccgagcgcgccggggtgcccgccttcctggagacctccgcgccccgcaacctccccttctacgagcggctcggcttcaccgtcaccgccgacgtcgaggtgcccgaaggaccgcgcacctggtgcatgacccgcaagcccggtgcctgaggtacctctcatgctggagttcttcgcccaccccaacttgtttattgcagcttataatggttacaaataaagcaatagcatcacaaatttcacaaataaagcatttttttcactgcattctagttgtggtttgtccaaactcatcaatgtatcttatcatcgatgaagttcctattctctagaaagtataggaacttctaacctcccgggtgacagataacttcgtataatgtatgctatacgaagttatgtcgacgcggcgcgccgaattataatactaacattactgaagaaaatgcccaaaagatggtaagttcttgaggctacccagggggttattgattgcttcttaaagatcagaattactgcctataaaactggataaggaaatcatagagatctctcaagtgtgaggatgagtgactgcctctgtagctctgatcctagtctcccagatggctaaattcaattgaccttagagttcatctggaaaattgttatgaatgaattatttgcccagattccaaagatgagtgaaaatgtttaataaagttgccatcactattctcattatatttggtatgtaaagcattcatggaaatgttctaagtcgttattgagccaataattttctttagcttataatgccaacaggtctatccgagaactacaaatgacatattaactgaaaaatgcaactggggtttactgaaggcagcagcttagtaattaaggtaaccatggcttaggtgaaactggacctgggaattccttctttcattgacacagagctctgaggaatttccaaaggtcacagaagaaaagctataattaaactagtcccaaaaaatctcagcctactctgggaaagcagcatattttgtttgacaagtgcaaggacttagaacttttttttttctcactgatcctgaagtgccttttaagtatagttaagtggtggaaaattgagcaactatttaagaaaagactcttttttttcttcttccagcaatgctttccttcaaaacggtagcttcaaaacttcctgtcttttaaatgatcagggggctgtgtgtttaaattattgccattcatagaacagagtgggtctgaggatgcctgtttcctttgaaattctatgccccctcccagttttctaaaatttaagaaaccacagagactttgacaatgtagttgccaaatgagttgcttttaactgctctaatagtttggtcttaagcttggcgtaatcatggtcatagctgtttcctgtgtgaaattgttatccgctcacaattccacacaacatacgagccggaagcataaagtgtaaagcctggggtgcctaatgagtgagctaactcacattaattgcgttgcgctcactgcccgctttccagtcgggaaacctgtcgtgccagctgcattaatgaatcggccaacgcgcggggagaggcggtttgcgtattgggcgctcttccgcttcctcgctcactgactcgctgcgctcggtcgttcggctgcggcgagcggtatcagctcactcaaaggcggtaatacggttatccacagaatcaggggataacgcaggaaagaacatgtgagcaaaaggccagcaaaaggccaggaaccgtaaaaaggccgcgttgctggcgtttttccataggctccgcccccctgacgagcatcacaaaaatcgacgctcaagtcagaggtggcgaaacccgacaggactataaagataccaggcgtttccccctggaagctccctcgtgcgctctcctgttccgaccctgccgcttaccggatacctgtccgcctttctcccttcgggaagcgtggcgctttctcatagctcacgctgtaggtatctcagttcggtgtaggtcgttcgctccaagctgggctgtgtgcacgaaccccccgttcagcccgaccgctgcgccttatccggtaactatcgtcttgagtccaacccggtaagacacgacttatcgccactggcagcagccactggtaacaggattagcagagcgaggtatgtaggcggtgctacagagttcttgaagtggtggcctaactacggctacactagaagaacagtatttggtatctgcgctctgctgaagccagttaccttcggaaaaagagttggtagctcttgatccggcaaacaaaccaccgctggtagcggtggtttttttgtttgcaagcagcagattacgcgcagaaaaaaaggatctcaagaagatcctttgatcttttctacggggtctgacgctcagtggaacgaaaactcacgttaagggattttggtcatgagattatcaaaaaggatcttcacctagatccttttaaattaaaaatgaagttttaaatcaatctaaagtatatatgagtaaacttggtctgacagttaccaatgcttaatcagtgaggcacctatctcagcgatctgtctatttcgttcatccatagttgcctgactccccgtcgtgtagataactacgatacgggagggcttaccatctggccccagtgctgcaatgataccgcgagacccacgctcaccggctccagatttatcagcaataaaccagccagccggaagggccgagcgcagaagtggtcctgcaactttatccgcctccatccagtctattaattgttgccgggaagctagagtaagtagttcgccagttaatagtttgcgcaacgttgttgccattgctacaggcatcgtggtgtcacgctcgtcgtttggtatggcttcattcagctccggttcccaacgatcaaggcgagttacatgatcccccatgttgtgcaaaaaagcggttagctccttcggtcctccgatcgttgtcagaagtaagttggccgcagtgttatcactcatggttatggcagcactgcataattctcttactgtcatgccatccgtaagatgcttttctgtgactggtgagtactcaaccaagtcattctgagaatagtgtatgcggcgaccgagttgctcttgcccggcgtcaatacgggataataccgcgccacatagcagaactttaaaagtgctcatcattggaaaacgttcttcggggcgaaaactctcaaggatcttaccgctgttgagatccagttcgatgtaacccactcgtgcacccaactgatcttcagcatcttttactttcaccagcgtttctgggtgagcaaaaacaggaaggcaaaatgccgcaaaaaagggaataagggcgacacggaaatgttgaatactcatactcttcctttttcaatattattgaagcatttatcagggttattgtctcatgagcggatacatatttgaatgtatttagaaaaataaacaaataggggttccgcgcacatttccccgaaaagtgccacctgacgtctaagaaaccattattatcatgacattaacctataaaaataggcgtatcacgaggccctttcgtc

SEQ ID NO: 28 - DNA, 19 bp, Natural sequence
  Puro-F
aacctccccttctacgagc

SEQ ID NO: 29 - DNA, 24 bp, Natural sequence
  3arm-outR
tacagccaggatctggatgtcagc

SEQ ID NO: 30 - DNA, 5922 bp, Artificial Sequence
  ACE2 genomic Replacing sequence of mouse embryonic stem cells
ccctatggagtggagaagagtcttataattttttaaatgggcagagaaatgaatttatttttaatttttagagacagggtttctttgtatagctctagctgtctttgattggtagacaaagctgtcctcaaactcagagatcttccttcctttgtctcctgagtgctgggattaaaggcatggaccaccactgccctgccccattctctccattaattttaagtgaatgcttgcaaaagctcacttctttggtgaacagcttcctttacaaataagtacctttgccttcgtttttataggattcttaaaaagaaaaaaaagattcagccaggtggttgtggtgcacacctttaatcccagcagtcaggaggcagaggaaagcagatctcttgagtttgaggctagcctagtctacagagggagttccaggacagccaaggctacagagaggaactgtctaaaaacaccaagaaagagagaaaggagagagggagaggatggatagcttattgatagaattgtcagaaaaggctataagttccaatatgtgtcccatgatttctaagtctagccctttctgttatagtaaaatcatagtacaccctcctcctccagtgtatctttaacagcttttaaggaacatattaactaaatgtccaggttttgatttggccataaaatgttagcaaagctaaggttttctaggattaatgaataacatgtctttatttagtttacttaaaaaaatcattctaaaatatctgtttacatatctgtcctctccaggattaacttcatattggtccagcagcttgtttactgttctcttctgtttcttcttctgctttttttttcttctcttctcagtgcccaacccaagttcaaaggctgatgagagagaaaaactcatgaagagattttactctagggaaagttgctcagtggatgggatcttggcgcacggggaaagatgtcaagctcttcctggctccttctcagccttgttgctgtaactgctgctcagtccaccattgaggaacaggccaagacatttttggacaagtttaaccacgaagccgaagacctgttctatcaaagttcacttgcttcttggaattataacaccaatattactgaagagaatgtccaaaacatgaataatgctggggacaaatggtctgcctttttaaaggaacagtccacacttgcccaaatgtatccactacaagaaattcagaatctcacagtcaagcttcagctgcaggctcttcagcaaaatgggtcttcagtgctctcagaagacaagagcaaacggttgaacacaattctaaatacaatgagcaccatctacagtactggaaaagtttgtaacccagataatccacaagaatgcttattacttgaaccaggtttgaatgaaataatggcaaacagtttagactacaatgagaggctctgggcttgggaaagctggagatctgaggtcggcaagcagctgaggccattatatgaagagtatgtggtcttgaaaaatgagatggcaagagcaaatcattatgaggactatggggattattggagaggagactatgaagtaaatggggtagatggctatgactacagccgcggccagttgattgaagatgtggaacatacctttgaagagattaaaccattatatgaacatcttcatgcctatgtgagggcaaagttgatgaatgcctatccttcctatatcagtccaattggatgcctccctgctcatttgcttggtgatatgtggggtagattttggacaaatctgtactctttgacagttccctttggacagaaaccaaacatagatgttactgatgcaatggtggaccaggcctgggatgcacagagaatattcaaggaggccgagaagttctttgtatctgttggtcttcctaatatgactcaaggattctgggaaaattccatgctaacggacccaggaaatgttcagaaagcagtctgccatcccacagcttgggacctggggaagggcgacttcaggatccttatgtgcacaaaggtgacaatggacgacttcctgacagctcatcatgagatggggcatatccagtatgatatggcatatgctgcacaaccttttctgctaagaaatggagctaatgaaggattccatgaagctgttggggaaatcatgtcactttctgcagccacacctaagcatttaaaatccattggtcttctgtcacccgattttcaagaagacaatgaaacagaaataaacttcctgctcaaacaagcactcacgattgttgggactctgccatttacttacatgttagagaagtggaggtggatggtctttaaaggggaaattcccaaagaccagtggatgaaaaagtggtgggagatgaagcgagagatagttggggtggtggaacctgtgccccatgatgaaacatactgtgaccccgcatctctgttccatgtttctaatgattactcattcattcgatattacacaaggaccctttaccaattccagtttcaagaagcactttgtcaagcagctaaacatgaaggccctctgcacaaatgtgacatctcaaactctacagaagctggacagaaactgttcaatatgctgaggcttggaaaatcagaaccctggaccctagcattggaaaatgttgtaggagcaaagaacatgaatgtaaggccactgctcaactactttgagcccttatttacctggctgaaagaccagaacaagaattcttttgtgggatggagtaccgactggagtccatatgcagaccaaagcatcaaagtgaggataagcctaaaatcagctcttggagataaagcatatgaatggaacgacaatgaaatgtacctgttccgatcatctgttgcatatgctatgaggcagtactttttaaaagtaaaaaatcagatgattctttttggggaggaggatgtgcgagtggctaatttgaaaccaagaatctcctttaatttctttgtcactgcacctaaaaatgtgtctgatatcattcctagaactgaagttgaaaaggccatcaggatgtcccggagccgtatcaatgatgctttccgtctgaatgacaacagcctagagtttctggggatacagccaacacttggacctcctaaccagccccctgtttccatatggctgattgtttttggagttgtgatgggagtgatagtggttggcattgtcatcctgatcttcactgggatcagagatcggaagaagaaaaataaagcaagaagtggagaaaatccttatgcctccatcgatattagcaaaggagaaaataatccaggattccaaaacactgatgatgttcagacctccttttagaacttgtttattgcagcttataatggttacaaataaagcaatagcatcacaaatttcacaaataaagcatttttttcactgcattctagttgtggtttgtccaaactcatcaatgtatcttaacgcgtgcgaagttcctattctctagaaagtataggaacttcatcgataccgggtaggggaggcgcttttcccaaggcagtctggagcatgcgctttagcagccccgctgggcacttggcgctacacaagtggcctctggcctcgcacacattccacatcccccggtaggcgccaaccggctccgttctttggtggccccttcgcgccaccttctactcctcccctagtcaggaagttcccccccgccccgcagctcgcgtcgtgcaggacgtgacaaatggaagtagcacgtctcactagtctcgtgcagatggacagcaccgctgagcaatggaagcgggtaggcctttggggcagcggccaatagcagctttgctccttcgctttctgggctcagaggctgggaaggggtgggtccgggggcgggctcaggggcgggctcaggggcggggcgggcgcccgaaggtcctccggaggcccggcattctgcacgcttcaaaagcgcacgtctgccgcgctgttctcctcttcctcatctccgggcctttcgacctgcagcccaagctagcttaccatgaccgagtacaagcccacggtgcgcctcgccacccgcgacgacgtccccagggccgtacgcaccctcgccgccgcgttcgccgactaccccgccacgcgccacaccgtcgatccggaccgccacatcgagcgggtcaccgagctgcaagaactcttcctcacgcgcgtcgggctcgacatcggcaaggtgtgggtcgcggacgacggcgccgcggtggcggtctggaccacgccggagagcgtcgaagcgggggcggtgttcgccgagatcggcccgcgcatggccgagttgagcggttcccggctggccgcgcagcaacagatggaaggcctcctggcgccgcaccggcccaaggagcccgcgtggttcctggccaccgtcggcgtctcgcccgaccaccagggcaagggtctgggcagcgccgtcgtgctccccggagtggaggcggccgagcgcgccggggtgcccgccttcctggagacctccgcgccccgcaacctccccttctacgagcggctcggcttcaccgtcaccgccgacgtcgaggtgcccgaaggaccgcgcacctggtgcatgacccgcaagcccggtgcctgaggtacctctcatgctggagttcttcgcccaccccaacttgtttattgcagcttataatggttacaaataaagcaatagcatcacaaatttcacaaataaagcatttttttcactgcattctagttgtggtttgtccaaactcatcaatgtatcttatcatcgatgaagttcctattctctagaaagtataggaacttctaacctcccgggtgacagataacttcgtataatgtatgctatacgaagttatgtcgacgcggcgcgccgaattataatactaacattactgaagaaaatgcccaaaagatggtaagttcttgaggctacccagggggttattgattgcttcttaaagatcagaattactgcctataaaactggataaggaaatcatagagatctctcaagtgtgaggatgagtgactgcctctgtagctctgatcctagtctcccagatggctaaattcaattgaccttagagttcatctggaaaattgttatgaatgaattatttgcccagattccaaagatgagtgaaaatgtttaataaagttgccatcactattctcattatatttggtatgtaaagcattcatggaaatgttctaagtcgttattgagccaataattttctttagcttataatgccaacaggtctatccgagaactacaaatgacatattaactgaaaaatgcaactggggtttactgaaggcagcagcttagtaattaaggtaaccatggcttaggtgaaactggacctgggaattccttctttcattgacacagagctctgaggaatttccaaaggtcacagaagaaaagctataattaaactagtcccaaaaaatctcagcctactctgggaaagcagcatattttgtttgacaagtgcaaggacttagaacttttttttttctcactgatcctgaagtgccttttaagtatagttaagtggtggaaaattgagcaactatttaagaaaagactcttttttttcttcttccagcaatgctttccttcaaaacggtagcttcaaaacttcctgtcttttaaatgatcagggggctgtgtgtttaaattattgccattcatagaacagagtgggtctgaggatgcctgtttcctttgaaattctatgccccctcccagttttctaaaatttaagaaaccacagagactttgacaatgtagttgccaaatgagttgcttttaactgctctaatagtttggtctt

SEQ ID NO: 31 - DNA, 19 bp, Natural sequence
  hACE2-F
tgatagtggttggcattgt

SEQ ID NO: 32 - DNA, 4591 bp, Artificial Sequence
  ACE2 genomic replacing sequence of mouse embryonic stem cells after removing PGK-puro
ccctatggagtggagaagagtcttataattttttaaatgggcagagaaatgaatttatttttaatttttagagacagggtttctttgtatagctctagctgtctttgattggtagacaaagctgtcctcaaactcagagatcttccttcctttgtctcctgagtgctgggattaaaggcatggaccaccactgccctgccccattctctccattaattttaagtgaatgcttgcaaaagctcacttctttggtgaacagcttcctttacaaataagtacctttgccttcgtttttataggattcttaaaaagaaaaaaaagattcagccaggtggttgtggtgcacacctttaatcccagcagtcaggaggcagaggaaagcagatctcttgagtttgaggctagcctagtctacagagggagttccaggacagccaaggctacagagaggaactgtctaaaaacaccaagaaagagagaaaggagagagggagaggatggatagcttattgatagaattgtcagaaaaggctataagttccaatatgtgtcccatgatttctaagtctagccctttctgttatagtaaaatcatagtacaccctcctcctccagtgtatctttaacagcttttaaggaacatattaactaaatgtccaggttttgatttggccataaaatgttagcaaagctaaggttttctaggattaatgaataacatgtctttatttagtttacttaaaaaaatcattctaaaatatctgtttacatatctgtcctctccaggattaacttcatattggtccagcagcttgtttactgttctcttctgtttcttcttctgctttttttttcttctcttctcagtgcccaacccaagttcaaaggctgatgagagagaaaaactcatgaagagattttactctagggaaagttgctcagtggatgggatcttggcgcacggggaaagatgtcaagctcttcctggctccttctcagccttgttgctgtaactgctgctcagtccaccattgaggaacaggccaagacatttttggacaagtttaaccacgaagccgaagacctgttctatcaaagttcacttgcttcttggaattataacaccaatattactgaagagaatgtccaaaacatgaataatgctggggacaaatggtctgcctttttaaaggaacagtccacacttgcccaaatgtatccactacaagaaattcagaatctcacagtcaagcttcagctgcaggctcttcagcaaaatgggtcttcagtgctctcagaagacaagagcaaacggttgaacacaattctaaatacaatgagcaccatctacagtactggaaaagtttgtaacccagataatccacaagaatgcttattacttgaaccaggtttgaatgaaataatggcaaacagtttagactacaatgagaggctctgggcttgggaaagctggagatctgaggtcggcaagcagctgaggccattatatgaagagtatgtggtcttgaaaaatgagatggcaagagcaaatcattatgaggactatggggattattggagaggagactatgaagtaaatggggtagatggctatgactacagccgcggccagttgattgaagatgtggaacatacctttgaagagattaaaccattatatgaacatcttcatgcctatgtgagggcaaagttgatgaatgcctatccttcctatatcagtccaattggatgcctccctgctcatttgcttggtgatatgtggggtagattttggacaaatctgtactctttgacagttccctttggacagaaaccaaacatagatgttactgatgcaatggtggaccaggcctgggatgcacagagaatattcaaggaggccgagaagttctttgtatctgttggtcttcctaatatgactcaaggattctgggaaaattccatgctaacggacccaggaaatgttcagaaagcagtctgccatcccacagcttgggacctggggaagggcgacttcaggatccttatgtgcacaaaggtgacaatggacgacttcctgacagctcatcatgagatggggcatatccagtatgatatggcatatgctgcacaaccttttctgctaagaaatggagctaatgaaggattccatgaagctgttggggaaatcatgtcactttctgcagccacacctaagcatttaaaatccattggtcttctgtcacccgattttcaagaagacaatgaaacagaaataaacttcctgctcaaacaagcactcacgattgttgggactctgccatttacttacatgttagagaagtggaggtggatggtctttaaaggggaaattcccaaagaccagtggatgaaaaagtggtgggagatgaagcgagagatagttggggtggtggaacctgtgccccatgatgaaacatactgtgaccccgcatctctgttccatgtttctaatgattactcattcattcgatattacacaaggaccctttaccaattccagtttcaagaagcactttgtcaagcagctaaacatgaaggccctctgcacaaatgtgacatctcaaactctacagaagctggacagaaactgttcaatatgctgaggcttggaaaatcagaaccctggaccctagcattggaaaatgttgtaggagcaaagaacatgaatgtaaggccactgctcaactactttgagcccttatttacctggctgaaagaccagaacaagaattcttttgtgggatggagtaccgactggagtccatatgcagaccaaagcatcaaagtgaggataagcctaaaatcagctcttggagataaagcatatgaatggaacgacaatgaaatgtacctgttccgatcatctgttgcatatgctatgaggcagtactttttaaaagtaaaaaatcagatgattctttttggggaggaggatgtgcgagtggctaatttgaaaccaagaatctcctttaatttctttgtcactgcacctaaaaatgtgtctgatatcattcctagaactgaagttgaaaaggccatcaggatgtcccggagccgtatcaatgatgctttccgtctgaatgacaacagcctagagtttctggggatacagccaacacttggacctcctaaccagccccctgtttccatatggctgattgtttttggagttgtgatgggagtgatagtggttggcattgtcatcctgatcttcactgggatcagagatcggaagaagaaaaataaagcaagaagtggagaaaatccttatgcctccatcgatattagcaaaggagaaaataatccaggattccaaaacactgatgatgttcagacctccttttagaacttgtttattgcagcttataatggttacaaataaagcaatagcatcacaaatttcacaaataaagcatttttttcactgcattctagttgtggtttgtccaaactcatcaatgtatcttaacgcgtgcgaagttcctattctctagaaagtataggaacttctaacctcccgggtgacagataacttcgtataatgtatgctatacgaagttatgtcgacgcggcgcgccgaattataatactaacattactgaagaaaatgcccaaaagatggtaagttcttgaggctacccagggggttattgattgcttcttaaagatcagaattactgcctataaaactggataaggaaatcatagagatctctcaagtgtgaggatgagtgactgcctctgtagctctgatcctagtctcccagatggctaaattcaattgaccttagagttcatctggaaaattgttatgaatgaattatttgcccagattccaaagatgagtgaaaatgtttaataaagttgccatcactattctcattatatttggtatgtaaagcattcatggaaatgttctaagtcgttattgagccaataattttctttagcttataatgccaacaggtctatccgagaactacaaatgacatattaactgaaaaatgcaactggggtttactgaaggcagcagcttagtaattaaggtaaccatggcttaggtgaaactggacctgggaattccttctttcattgacacagagctctgaggaatttccaaaggtcacagaagaaaagctataattaaactagtcccaaaaaatctcagcctactctgggaaagcagcatattttgtttgacaagtgcaaggacttagaacttttttttttctcactgatcctgaagtgccttttaagtatagttaagtggtggaaaattgagcaactatttaagaaaagactcttttttttcttcttccagcaatgctttccttcaaaacggtagcttcaaaacttcctgtcttttaaatgatcagggggctgtgtgtttaaattattgccattcatagaacagagtgggtctgaggatgcctgtttcctttgaaattctatgccccctcccagttttctaaaatttaagaaaccacagagactttgacaatgtagttgccaaatgagttgcttttaactgctctaatagtttggtctt